European Patent Specification EP 3 750 552 B1, published May 10, 2023. Title: GDF TRAPS FOR USE TO TREAT ANEMIA. Applicant: ACCELERON PHARMA INC. The sequence listing filed with the application follows.

SEQUENCE LISTING (44 sequences)

SEQ ID NO: 1 - protein, 512 aa, Homo sapiens
MTAPWVALALLWGSLWPGSGRGEAETRECIYYNANWELERTNQSGLERCEGEQDKRLHCYASWRNSSGTIELVKKGCWLDDFNCYDRQECVATEENPQVYFCCCEGNFCNERFTHLPEAGGPEVTYEPPPTAPTLLTVLAYSLLPIGGLSLIVLLAFWMYRHRKPPYGHVDIHEDPGPPPPSPLVGLKPLQLLEIKARGRFGCVWKAQLMNDFVAVKIFPLQDKQSWQSEREIFSTPGMKHENLLQFIAAEKRGSNLEVELWLITAFHDKGSLTDYLKGNIITWNELCHVAETMSRGLSYLHEDVPWCRGEGHKPSIAHRDFKSKNVLLKSDLTAVLADFGLAVRFEPGKPPGDTHGQVGTRRYMAPEVLEGAINFQRDAFLRIDMYAMGLVLWELVSRCKAADGPVDEYMLPFEEEIGQHPSLEELQEVVVHKKMRPTIKDHWLKHPGLAQLCVTIEECWDHDAEARLSAGCVEERVSLIRRSVNGTTSDCLVSLVTSVTNVDLPPKESSI

SEQ ID NO: 2 - protein, 115 aa, Homo sapiens
GRGEAETRECIYYNANWELERTNQSGLERCEGEQDKRLHCYASWRNSSGTIELVKKGCWLDDFNCYDRQECVATEENPQVYFCCCEGNFCNERFTHLPEAGGPEVTYEPPPTAPT

SEQ ID NO: 3 - protein, 100 aa, Homo sapiens
GRGEAETRECIYYNANWELERTNQSGLERCEGEQDKRLHCYASWRNSSGTIELVKKGCWLDDFNCYDRQECVATEENPQVYFCCCEGNFCNERFTHLPEA

SEQ ID NO: 4 - DNA, 1539 bp, Homo sapiens
atgacggcgccctgggtggccctcgccctcctctggggatcgctgtggcccggctctgggcgtggggaggctgagacacgggagtgcatctactacaacgccaactgggagctggagcgcaccaaccagagcggcctggagcgctgcgaaggcgagcaggacaagcggctgcactgctacgcctcctgggccaacagctctggcaccatcgagctcgtgaagaagggctgctggctagatgacttcaactgctacgataggcaggagtgtgtggccactgaggagaacccccaggtgtacttctgctgctgtgaaggcaacttctgcaacgagcgcttcactcatttgccagaggctgggggcccggaagtcacgtacgagccacccccgacagcccccaccctgctcacggtgctggcctactcactgctgcccatcgggggcctttccctcatcgtcctgctggccttttggatgtaccggcatcgcaagcccccctacggtcatgtggacatccatgaggaccctgggcctccaccaccatcccctctggtgggcctgaagccactgcagctgctggagatcaaggctcgggggcgctttggctgtgtctggaaggcccagctcatgaatgactttgtagctgtcaagatcttcccactccaggacaagcagtcgtggcagagtgaacgggagatcttcagcacacctggcatgaagcacgagaacctgctacagttcattgctgccgagaagcgaggctccaacctcgaagtagagctgtggctcatcacggccttccatgacaagggctccctcacggattacctcaaggggaacatcatcacatggaacgaactgtgtcatgtagcagagacgatgtcacgaggcctctcatacctgcatgaggatgtgccctggtgccgtggcgagggccacaagccgtctattgcccacagggactttaaaagtaagaatgtattgctgaagagcgacctcacagccgtgctggctgactttggcttggctgttcgatttgagccagggaaacctccaggggacacccacggacaggtaggcacgagacggtacatggctcctgaggtgctcgagggagccatcaacttccagagagatgccttcctgcgcattgacatgtatgccatggggttggtgctgtgggagcttgtgtctcgctgcaaggctgcagacggacccgtggatgagtacatgctgccctttgaggaagagattggccagcacccttcgttggaggagctgcaggaggtggtggtgcacaagaagatgaggcccaccattaaagatcactggttgaaacacccgggcctggcccagctttgtgtgaccatcgaggagtgctgggaccatgatgcagaggctcgcttgtccgcgggctgtgtggaggagcgggtgtccctgattcggaggtcggtcaacggcactacctcggactgtctcgtttccctggtgacctctgtcaccaatgtggacctgccccctaaagagtcaagcatctaa

SEQ ID NO: 5 - DNA, 345 bp, Homo sapiens
gggcgtggggaggctgagacacgggagtgcatctactacaacgccaactgggagctggagcgcaccaaccagagcggcctggagcgctgcgaaggcgagcaggacaagcggctgcactgctacgcctcctgggccaacagctctggcaccatcgagctcgtgaagaagggctgctggctagatgacttcaactgctacgataggcaggagtgtgtggccactgaggagaacccccaggtgtacttctgctgctgtgaaggcaacttctgcaacgagcgcttcactcatttgccagaggctgggggcccggaagtcacgtacgagccacccccgacagcccccacc

SEQ ID NO: 6 - protein, 225 aa, Artificial Sequence
  Description of Artificial Sequence: Synthetic polypeptide
  MOD_RES (43)..(43): Asp or Ala
  MOD_RES (100)..(100): Lys or Ala
  MOD_RES (212)..(212): Asn or Ala
THTCPPCPAPELLGGPSVFLFPPKPKDTLMISRTPEVTCVVVXVSHEDPEVKFNWYVDGVEVHNAKTKPREEQYNSTYRVVSVLTVLHQDWLNGKEYKCXVSNKALPVPIEKTISKAKGQPREPQVYTLPPSREEMTKNQVSLTCLVKGFYPSDIAVEWESNGQPENNYKTTPPVLDSDGPFFLYSKLTVDKSRWQQGNVFSCSVMHEALHXHYTQKSLSLSPGK

SEQ ID NO: 7 - protein, 343 aa, Artificial Sequence
  Description of Artificial Sequence: Synthetic polypeptide
GRGEAETRECIYYNANWELERTNQSGLERCEGEQDKRLHCYASWRNSSGTIELVKKGCWDDDFNCYDRQECVATEENPQVYFCCCEGNFCNERFTHLPEAGGPEVTYEPPPTAPTGGGTHTCPPCPAPELLGGPSVFLFPPKPKDTLMISRTPEVTCVVVDVSHEDPEVKFNWYVDGVEVHNAKTKPREEQYNSTYRVVSVLTVLHQDWLNGKEYKCKVSNKALPVPIEKTISKAKGQPREPQVYTLPPSREEMTKNQVSLTCLVKGFYPSDIAVEWESNGQPENNYKTTPPVLDSDGSFFLYSKLTVDKSRWQQGNVFSCSVMHEALHNHYTQKSLSLSPGK

SEQ ID NO: 8 - protein, 21 aa, Apis mellifera
MKFLVNVALVFMVVYISYIYA

SEQ ID NO: 9 - protein, 22 aa, Unknown
  Description of Unknown: Tissue Plasminogen Activator
MDAMKRGLCCVLLLCGAVFVSP

SEQ ID NO: 10 - protein, 19 aa, Unknown
  Description of Unknown: Native peptide
MTAPWVALALLWGSLCAGS

SEQ ID NO: 11 - protein, 368 aa, Artificial Sequence
  Description of Artificial Sequence: Synthetic polypeptide
MDAMKRGLCCVLLLCGAVFVSPGASGRGEAETRECIYYNANWELERTNQSGLERCEGEQDKRLHCYASWRNSSGTIELVKKGCWDDDFNCYDRQECVATEENPQVYFCCCEGNFCNERFTHLPEAGGPEVTYEPPPTAPTGGGTHTCPPCPAPELLGGPSVFLFPPKPKDTLMISRTPEVTCVVVDVSHEDPEVKFNWYVDGVEVHNAKTKPREEQYNSTYRVVSVLTVLHQDWLNGKEYKCKVSNKALPVPIEKTISKAKGQPREPQVYTLPPSREEMTKNQVSLTCLVKGFYPSDIAVEWESNGQPENNYKTTPPVLDSDGSFFLYSKLTVDKSRWQQGNVFSCSVMHEALHNHYTQKSLSLSPGK

SEQ ID NO: 12 - DNA, 1107 bp, Artificial Sequence
  Description of Artificial Sequence: Synthetic polynucleotide
atggatgcaatgaagagagggctctgctgtgtgctgctgctgtgtggagcagtcttcgtttcgcccggcgcctctgggcgtggggaggctgagacacgggagtgcatctactacaacgccaactgggagctggagcgcaccaaccagagcggcctggagcgctgcgaaggcgagcaggacaagcggctgcactgctacgcctcctggcgcaacagctctggcaccatcgagctcgtgaagaagggctgctgggacgatgacttcaactgctacgataggcaggagtgtgtggccactgaggagaacccccaggtgtacttctgctgctgtgaaggcaacttctgcaacgagcgcttcactcatttgccagaggctgggggcccggaagtcacgtacgagccacccccgacagcccccaccggtggtggaactcacacatgcccaccgtgcccagcacctgaactcctggggggaccgtcagtcttcctcttccccccaaaacccaaggacaccctcatgatctcccggacccctgaggtcacatgcgtggtggtggacgtgagccacgaagaccctgaggtcaagttcaactggtacgtggacggcgtggaggtgcataatgccaagacaaagccgcgggaggagcagtacaacagcacgtaccgtgtggtcagcgtcctcaccgtcctgcaccaggactggctgaatggcaaggagtacaagtgcaaggtctccaacaaagccctcccagtccccatcgagaaaaccatctccaaagccaaagggcagccccgagaaccacaggtgtacaccctgcccccatcccgggaggagatgaccaagaaccaggtcagcctgacctgcctggtcaaaggcttctatcccagcgacatcgccgtggagtgggagagcaatgggcagccggagaacaactacaagaccacgcctcccgtgctggactccgacggctccttcttcctctatagcaagctcaccgtggacaagagcaggtggcagcaggggaacgtcttctcatgctccgtgatgcatgaggctctgcacaaccactacacgcagaagagcctctccctgtctccgggtaaatga

SEQ ID NO: 13 - protein, 5 aa, Artificial Sequence
  Description of Artificial Sequence: Synthetic peptide
TGGGG

SEQ ID NO: 14 - protein, 5 aa, Artificial Sequence
  Description of Artificial Sequence: Synthetic peptide
SGGGG

SEQ ID NO: 15 - protein, 116 aa, Homo sapiens
ILGRSETQECLFFNANWEKDRTNQTGVEPCYGDKDKRRHCFATWKNISGSIEIVKQGCWLDDINCYDRTDCVEKKDSPEVYFCCCEGNMCNEKFSYFPEMEVTQPTSNPVTPKPPT

SEQ ID NO: 16 - protein, 150 aa, Rattus sp.
MTAPWAALALLWGSLCAGSGRGEAETRECIYYNANWELERTNQSGLERCEGEQDKRLHCYASWPNSSGTIELVKKGCWLDDFNCYDRQECVATEENPQVYFCCCEGNFCNERFTHLPEPGGPEVTYEPPPTAPTLLTVLAYSLLPIGGLS

SEQ ID NO: 17 - protein, 150 aa, Sus sp.
MTAPWAALALLWGSLCVGSGRGEAETRECIYYNANWELERTNQSGLERCEGEQDKRLHCYASWRNSSGTIELVKKGCWLDDFNCYDRQECVATEENPQVYFCCCEGNFCNERFTHLPEAGGPEVTYEPPPTAPTLLTVLAYSLLPIGGLS

SEQ ID NO: 18 - protein, 150 aa, Mus sp.
MTAPWAALALLWGSLCAGSGRGEAETRECIYYNANWELERTNQSGLERCEGEQDKRLHCYASWRNSSGTIELVKKGCWLDDFNCYDRQECVATEENPQVYFCCCEGNFCNERFTHLPEPGGPEVTYEPPPTAPTLLTVLAYSLLPIGGLS

SEQ ID NO: 19 - protein, 150 aa, Homo sapiens
MTAPWVALALLWGSLCAGSGRGEAETRECIYYNANWELERTNQSGLERCEGEQDKRLHCYASWRNSSGTIELVKKGCWLDDFNCYDRQECVATEENPQVYFCCCEGNFCNERFTHLPEAGGPEVTYEPPPTAPTLLTVLAYSLLPIGGLS

SEQ ID NO: 20 - protein, 150 aa, Bos sp.
MTAPWAALALLWGSLCAGSGRGEAETRECIYYNANWELERTNQSGLERCEGERDKRLHCYASWRNSSGTIELVKKGCWLDDFNCYDRQECVATEENPQVYFCCCEGNFCNERFTHLPEAGGPEVTYEPPPTAPTLLTVLAYSLLPVGGLS

SEQ ID NO: 21 - protein, 150 aa, Xenopus sp.
MGASVALTFLLLLATFRAGSGHDEVETRECIYYNANWELEKTNQSGVERLVEGKKDKRLHCYASWRNNSGFIELVKKGCWLDDFNCYDRQECIAKEENPQVFFCCCEGNYCNKKFTHLPEVETFDPKPQPSASVLNILIYSLLPIVGLSM

SEQ ID NO: 22 - protein, 150 aa, Homo sapiens
MGAAAKLAFAVFLISCSSGAILGRSETQECLFFNANWEKDRTNQTGVEPCYGDKDKRRHCFATWKNISGSIEIVKQGCWLDDINCYDRTDCVEKKDSPEVYFCCCEGNMCNEKFSYFPEMEVTQPTSNPVTPKPPYYNILLYSLVPLMLI

SEQ ID NO: 23 - protein, 154 aa, Artificial Sequence
  Description of Artificial Sequence: Synthetic consensus polypeptide
  MOD_RES (8)..(8): Thr or Ala
  MOD_RES (121)..(121): Pro, Ala, Val or Met
MTAPWAAXLALLWGSLCAGSGRGEAETRECIYYNANWELERTNQSGLERLCEGEQDKRLHCYASWRNSSGTLELVKKGCWLDDFNCYDRQECVATEENPQVYFCCCEGNFCNERFTHLPEXGGPEVTYEPKPPTAPTLLTVLAYSLLPIGGLSM

SEQ ID NO: 24 - protein, 6 aa, Artificial Sequence
  Description of Artificial Sequence: Synthetic 6xHis tag
HHHHHH

SEQ ID NO: 25 - DNA, 1107 bp, Artificial Sequence
  Description of Artificial Sequence: Synthetic polynucleotide
atggatgcaatgaagagagggctctgctgtgtgctgctgctgtgtggagcagtcttcgtttcgcccggcgcctctgggcgtggggaggctgagacacgggagtgcatctactacaacgccaactgggagctggagcgcaccaaccagagcggcctggagcgctgcgaaggcgagcaggacaagcggctgcactgctacgcctcctggcgcaacagctctggcaccatcgagctcgtgaagaagggctgctgggatgatgacttcaactgctacgataggcaggagtgtgtggccactgaggagaacccccaggtgtacttctgctgctgtgaaggcaacttctgcaacgagcgcttcactcatttgccagaggctgggggcccggaagtcacgtacgagccacccccgacagcccccaccggtggtggaactcacacatgcccaccgtgcccagcacctgaactcctggggggaccgtcagtcttcctcttccccccaaaacccaaggacaccctcatgatctcccggacccctgaggtcacatgcgtggtggtggacgtgagccacgaagaccctgaggtcaagttcaactggtacgtggacggcgtggaggtgcataatgccaagacaaagccgcgggaggagcagtacaacagcacgtaccgtgtggtcagcgtcctcaccgtcctgcaccaggactggctgaatggcaaggagtacaagtgcaaggtctccaacaaagccctcccagcccccatcgagaaaaccatctccaaagccaaagggcagccccgagaaccacaggtgtacaccctgcccccatcccgggaggagatgaccaagaaccaggtcagcctgacctgcctggtcaaaggcttctatcccagcgacatcgccgtggagtgggagagcaatgggcagccggagaacaactacaagaccacgcctcccgtgctggactccgacggctccttcttcctctatagcaagctcaccgtggacaagagcaggtggcagcaggggaacgtcttctcatgctccgtgatgcatgaggctctgcacaaccactacacgcagaagagcctctccctgtccccgggtaaatga

SEQ ID NO: 26 - protein, 360 aa, Artificial Sequence
  Description of Artificial Sequence: Synthetic polypeptide
MDAMKRGLCCVLLLCGAVFVSPGAAETRECIYYNANWELERTNQSGLERCEGEQDKRLHCYASWRNSSGTIELVKKGCWDDDFNCYDRQECVATEENPQVYFCCCEGNFCNERFTHLPEAGGPEVTYEPPPTGGGTHTCPPCPAPELLGGPSVFLFPPKPKDTLMISRTPEVTCVVVDVSHEDPEVKFNWYVDGVEVHNAKTKPREEQYNSTYRVVSVLTVLHQDWLNGKEYKCKVSNKALPAPIEKTISKAKGQPREPQVYTLPPSREEMTKNQVSLTCLVKGFYPSDIAVEWESNGQPENNYKTTPPVLDSDGSFFLYSKLTVDKSRWQQGNVFSCSVMHEALHNHYTQKSLSLSPGK

SEQ ID NO: 27 - DNA, 1083 bp, Artificial Sequence
  Description of Artificial Sequence: Synthetic polynucleotide
  CDS (76)..(396)
atggatgcaatgaagagagggctctgctgtgtgctgctgctgtgtggagcagtcttcgtttcgcccggcgccgctgagacacgggagtgcatctactacaacgccaactgggagctggagcgcaccaaccagagcggcctggagcgctgcgaaggcgagcaggacaagcggctgcactgctacgcctcctggcgcaacagctctggcaccatcgagctcgtgaagaagggctgctgggacgatgacttcaactgctacgataggcaggagtgtgtggccactgaggagaacccccaggtgtacttctgctgctgtgaaggcaacttctgcaacgagcgcttcactcatttgccagaggctgggggcccggaagtcacgtacgagccacccccgacaggtggtggaactcacacatgcccaccgtgcccagcacctgaactcctggggggaccgtcagtcttcctcttccccccaaaacccaaggacaccctcatgatctcccggacccctgaggtcacatgcgtggtggtggacgtgagccacgaagaccctgaggtcaagttcaactggtacgtggacggcgtggaggtgcataatgccaagacaaagccgcgggaggagcagtacaacagcacgtaccgtgtggtcagcgtcctcaccgtcctgcaccaggactggctgaatggcaaggagtacaagtgcaaggtctccaacaaagccctcccagcccccatcgagaaaaccatctccaaagccaaagggcagccccgagaaccacaggtgtacaccctgcccccatcccgggaggagatgaccaagaaccaggtcagcctgacctgcctggtcaaaggcttctatcccagcgacatcgccgtggagtgggagagcaatgggcagccggagaacaactacaagaccacgcctcccgtgctggactccgacggctccttcttcctctatagcaagctcaccgtggacaagagcaggtggcagcaggggaacgtcttctcatgctccgtgatgcatgaggctctgcacaaccactacacgcagaagagcctctccctgtccccgggtaaatga

SEQ ID NO: 28 - protein, 335 aa, Artificial Sequence
  Description of Artificial Sequence: Synthetic polypeptide
ETRECIYYNANWELERTNQSGLERCEGEQDKRLHCYASWRNSSGTIELVKKGCWDDDFNCYDRQECVATEENPQVYFCCCEGNFCNERFTHLPEAGGPEVTYEPPPTGGGTHTCPPCPAPELLGGPSVFLFPPKPKDTLMISRTPEVTCVVVDVSHEDPEVKFNWYVDGVEVHNAKTKPREEQYNSTYRVVSVLTVLHQDWLNGKEYKCKVSNKALPAPIEKTISKAKGQPREPQVYTLPPSREEMTKNQVSLTCLVKGFYPSDIAVEWESNGQPENNYKTTPPVLDSDGSFFLYSKLTVDKSRWQQGNVFSCSVMHEALHNHYTQKSLSLSPGK

SEQ ID NO: 29 - protein, 107 aa, Artificial Sequence
  Description of Artificial Sequence: Synthetic polypeptide
ETRECIYYNANWELERTNQSGLERCEGEQDKRLHCYASWRNSSGTIELVKKGCWDDDFNCYDRQECVATEENPQVYFCCCEGNFCNERFTHLPEAGGPEVTYEPPPT

SEQ ID NO: 30 - DNA, 1083 bp, Artificial Sequence
  Description of Artificial Sequence: Synthetic polynucleotide
  CDS (76)..(396)
atggatgcaatgaagagagggctctgctgtgtgctgctgctgtgtggagcagtcttcgtttcgcccggcgccgccgaaacccgcgaatgtatttattacaatgctaattgggaactcgaacggacgaaccaatccgggctcgaacggtgtgagggggaacaggataaacgcctccattgctatgcgtcgtggaggaactcctccgggacgattgaactggtcaagaaagggtgctgggacgacgatttcaattgttatgaccgccaggaatgtgtcgcgaccgaagagaatccgcaggtctatttctgttgttgcgaggggaatttctgtaatgaacggtttacccacctccccgaagccggcgggcccgaggtgacctatgaacccccgcccaccggtggtggaactcacacatgcccaccgtgcccagcacctgaactcctggggggaccgtcagtcttcctcttccccccaaaacccaaggacaccctcatgatctcccggacccctgaggtcacatgcgtggtggtggacgtgagccacgaagaccctgaggtcaagttcaactggtacgtggacggcgtggaggtgcataatgccaagacaaagccgcgggaggagcagtacaacagcacgtaccgtgtggtcagcgtcctcaccgtcctgcaccaggactggctgaatggcaaggagtacaagtgcaaggtctccaacaaagccctcccagcccccatcgagaaaaccatctccaaagccaaagggcagccccgagaaccacaggtgtacaccctgcccccatcccgggaggagatgaccaagaaccaggtcagcctgacctgcctggtcaaaggcttctatcccagcgacatcgccgtggagtgggagagcaatgggcagccggagaacaactacaagaccacgcctcccgtgctggactccgacggctccttcttcctctatagcaagctcaccgtggacaagagcaggtggcagcaggggaacgtcttctcatgctccgtgatgcatgaggctctgcacaaccactacacgcagaagagcctctccctgtccccgggtaaatga

SEQ ID NO: 31 - DNA, 321 bp, Artificial Sequence
  Description of Artificial Sequence: Synthetic polynucleotide
gaaacccgcgaatgtatttattacaatgctaattgggaactcgaacggacgaaccaatccgggctcgaacggtgtgagggggaacaggataaacgcctccattgctatgcgtcgtggaggaactcctccgggacgattgaactggtcaagaaagggtgctgggacgacgatttcaattgttatgaccgccaggaatgtgtcgcgaccgaagagaatccgcaggtctatttctgttgttgcgaggggaatttctgtaatgaacggtttacccacctccccgaagccggcgggcccgaggtgacctatgaacccccgcccacc

SEQ ID NO: 32 - protein, 115 aa, Homo sapiens
GRGEAETRECIYYNANWELERTNQSGLERCEGEQDKRLHCYASWRNSSGTIELVKKGCWDDDFNCYDRQECVATEENPQVYFCCCEGNFCNERFTHLPEAGGPEVTYEPPPTAPT

SEQ ID NO: 33 - DNA, 1107 bp, Artificial Sequence
  Description of Artificial Sequence: Synthetic polynucleotide
tacctacgttacttctctcccgagacgacacacgacgacgacacacctcgtcagaagcaaagcgggccgcggagacccgcacccctccgactctgtgccctcacgtagatgatgttgcggttgaccctcgacctcgcgtggttggtctcgccggacctcgcgacgcttccgctcgtcctgttcgccgacgtgacgatgcggaggaccgcgttgtcgagaccgtggtagctcgagcacttcttcccgacgaccctactactgaagttgacgatgctatccgtcctcacacaccggtgactcctcttgggggtccacatgaagacgacgacacttccgttgaagacgttgctcgcgaagtgagtaaacggtctccgacccccgggccttcagtgcatgctcggtgggggctgtcgggggtggccaccaccttgagtgtgtacgggtggcacgggtcgtggacttgaggacccccctggcagtcagaaggagaaggggggttttgggttcctgtgggagtactagagggcctggggactccagtgtacgcaccaccacctgcactcggtgcttctgggactccagttcaagttgaccatgcacctgccgcacctccacgtattacggttctgtttcggcgccctcctcgtcatgttgtcgtgcatggcacaccagtcgcaggagtggcaggacgtggtcctgaccgacttaccgttcctcatgttcacgttccagaggttgtttcgggagggtcgggggtagctcttttggtagaggtttcggtttcccgtcggggctcttggtgtccacatgtgggacgggggtagggccctcctctactggttcttggtccagtcggactggacggaccagtttccgaagatagggtcgctgtagcggcacctcaccctctcgttacccgtcggcctcttgttgatgttctggtgcggagggcacgacctgaggctgccgaggaagaaggagatatcgttcgagtggcacctgttctcgtccaccgtcgtccccttgcagaagagtacgaggcactacgtactccgagacgtgttggtgatgtgcgtcttctcggagagggacaggggcccatttact

SEQ ID NO: 34 - DNA, 1083 bp, Artificial Sequence
  Description of Artificial Sequence: Synthetic polynucleotide
tacctacgttacttctctcccgagacgacacacgacgacgacacacctcgtcagaagcaaagcgggccgcggcgactctgtgccctcacgtagatgatgttgcggttgaccctcgacctcgcgtggttggtctcgccggacctcgcgacgcttccgctcgtcctgttcgccgacgtgacgatgcggaggaccgcgttgtcgagaccgtggtagctcgagcacttcttcccgacgaccctgctactgaagttgacgatgctatccgtcctcacacaccggtgactcctcttgggggtccacatgaagacgacgacacttccgttgaagacgttgctcgcgaagtgagtaaacggtctccgacccccgggccttcagtgcatgctcggtgggggctgtccaccaccttgagtgtgtacgggtggcacgggtcgtggacttgaggacccccctggcagtcagaaggagaaggggggttttgggttcctgtgggagtactagagggcctggggactccagtgtacgcaccaccacctgcactcggtgcttctgggactccagttcaagttgaccatgcacctgccgcacctccacgtattacggttctgtttcggcgccctcctcgtcatgttgtcgtgcatggcacaccagtcgcaggagtggcaggacgtggtcctgaccgacttaccgttcctcatgttcacgttccagaggttgtttcgggagggtcgggggtagctcttttggtagaggtttcggtttcccgtcggggctcttggtgtccacatgtgggacgggggtagggccctcctctactggttcttggtccagtcggactggacggaccagtttccgaagatagggtcgctgtagcggcacctcaccctctcgttacccgtcggcctcttgttgatgttctggtgcggagggcacgacctgaggctgccgaggaagaaggagatatcgttcgagtggcacctgttctcgtccaccgtcgtccccttgcagaagagtacgaggcactacgtactccgagacgtgttggtgatgtgcgtcttctcggagagggacaggggcccatttact

SEQ ID NO: 35 - DNA, 1083 bp, Artificial Sequence
  Description of Artificial Sequence: Synthetic polynucleotide
tacctacgttacttctctcccgagacgacacacgacgacgacacacctcgtcagaagcaaagcgggccgcggcggctttgggcgcttacataaataatgttacgattaacccttgagcttgcctgcttggttaggcccgagcttgccacactcccccttgtcctatttgcggaggtaacgatacgcagcacctccttgaggaggccctgctaacttgaccagttctttcccacgaccctgctgctaaagttaacaatactggcggtccttacacagcgctggcttctcttaggcgtccagataaagacaacaacgctccccttaaagacattacttgccaaatgggtggaggggcttcggccgcccgggctccactggatacttgggggcgggtggccaccaccttgagtgtgtacgggtggcacgggtcgtggacttgaggacccccctggcagtcagaaggagaaggggggttttgggttcctgtgggagtactagagggcctggggactccagtgtacgcaccaccacctgcactcggtgcttctgggactccagttcaagttgaccatgcacctgccgcacctccacgtattacggttctgtttcggcgccctcctcgtcatgttgtcgtgcatggcacaccagtcgcaggagtggcaggacgtggtcctgaccgacttaccgttcctcatgttcacgttccagaggttgtttcgggagggtcgggggtagctcttttggtagaggtttcggtttcccgtcggggctcttggtgtccacatgtgggacgggggtagggccctcctctactggttcttggtccagtcggactggacggaccagtttccgaagatagggtcgctgtagcggcacctcaccctctcgttacccgtcggcctcttgttgatgttctggtgcggagggcacgacctgaggctgccgaggaagaaggagatatcgttcgagtggcacctgttctcgtccaccgtcgtccccttgcagaagagtacgaggcactacgtactccgagacgtgttggtgatgtgcgtcttctcggagagggacaggggcccatttact

SEQ ID NO: 36 - protein, 141 aa, Homo sapiens
GRGEAETRECIYYNANWELERTNQSGLERCEGEQDKRLHCYASWRNSSGTIELVKKGCWLDDFNCYDRQECVATEENPQVYFCCCEGNFCNERFTHLPEAGGPEGPWASTTIPSGGPEATAAAGDQGSGALWLCLEGPAHE

SEQ ID NO: 37 - protein, 141 aa, Artificial Sequence
  Description of Artificial Sequence: Synthetic polypeptide
GRGEAETRECIYYNANWELERTNQSGLERCEGEQDKRLHCYASWRNSSGTIELVKKGCWDDDFNCYDRQECVATEENPQVYFCCCEGNFCNERFTHLPEAGGPEGPWASTTIPSGGPEATAAAGDQGSGALWLCLEGPAHE

SEQ ID NO: 38 - protein, 370 aa, Artificial Sequence
  Description of Artificial Sequence: Synthetic polypeptide
GRGEAETRECIYYNANWELERTNQSGLERCEGEQDKRLHCYASWRNSSGTIELVKKGCWDDDFNCYDRQECVATEENPQVYFCCCEGNFCNERFTHLPEAGGPEGPWASTTIPSGGPEATAAAGDQGSGALWLCLEGPAHETGGGTHTCPPCPAPELLGGPSVFLFPPKPKDTLMISRTPEVTCVVVDVSHEDPEVKFNWYVDGVEVHNAKTKPREEQYNSTYRVVSVLTVLHQDWLNGKEYKCKVSNKALPAPIEKTISKAKGQPREPQVYTLPPSREEMTKNQVSLTCLVKGFYPSDIAVEWESNGQPENNYKTTPPVLDSDGSFFLYSKLTVDKSRWQQGNVFSCSVMHEALHNHYTQKSLSLSPGK

SEQ ID NO: 39 - protein, 512 aa, Homo sapiens
MTAPWVALALLWGSLWPGSGRGEAETRECIYYNANWELERTNQSGLERCEGEQDKRLHCYASWANSSGTIELVKKGCWLDDFNCYDRQECVATEENPQVYFCCCEGNFCNERFTHLPEAGGPEVTYEPPPTAPTLLTVLAYSLLPIGGLSLIVLLAFWMYRHRKPPYGHVDIHEDPGPPPPSPLVGLKPLQLLEIKARGRFGCVWKAQLMNDFVAVKIFPLQDKQSWQSEREIFSTPGMKHENLLQFIAAEKRGSNLEVELWLITAFHDKGSLTDYLKGNIITWNELCHVAETMSRGLSYLHEDVPWCRGEGHKPSIAHRDFKSKNVLLKSDLTAVLADFGLAVRFEPGKPPGDTHGQVGTRRYMAPEVLEGAINFQRDAFLRIDMYAMGLVLWELVSRCKAADGPVDEYMLPFEEEIGQHPSLEELQEVVVHKKMRPTIKDHWLKHPGLAQLCVTIEECWDHDAEARLSAGCVEERVSLIRRSVNGTTSDCLVSLVTSVTNVDLPPKESSI

SEQ ID NO: 40 - protein, 115 aa, Homo sapiens
GRGEAETRECIYYNANWELERTNQSGLERCEGEQDKRLHCYASWANSSGTIELVKKGCWLDDFNCYDRQECVATEENPQVYFCCCEGNFCNERFTHLPEAGGPEVTYEPPPTAPT

SEQ ID NO: 41 - protein, 100 aa, Homo sapiens
GRGEAETRECIYYNANWELERTNQSGLERCEGEQDKRLHCYASWANSSGTIELVKKGCWLDDFNCYDRQECVATEENPQVYFCCCEGNFCNERFTHLPEA

SEQ ID NO: 42 - protein, 4 aa, Artificial Sequence
  Description of Artificial Sequence: Synthetic peptide
TGGG

SEQ ID NO: 43 - protein, 368 aa, Artificial Sequence
  Description of Artificial Sequence: Synthetic polypeptide
MDAMKRGLCCVLLLCGAVFVSPGASGRGEAETRECIYYNANWELERTNQSGLERCEGEQDKRLHCYASWRNSSGTIELVKKGCWDDDFNCYDRQECVATEENPQVYFCCCEGNFCNERFTHLPEAGGPEVTYEPPPTAPTGGGTHTCPPCPAPELLGGPSVFLFPPKPKDTLMISRTPEVTCVVVDVSHEDPEVKFNWYVDGVEVHNAKTKPREEQYNSTYRVVSVLTVLHQDWLNGKEYKCKVSNKALPAPIEKTISKAKGQPREPQVYTLPPSREEMTKNQVSLTCLVKGFYPSDIAVEWESNGQPENNYKTTPPVLDSDGSFFLYSKLTVDKSRWQQGNVFSCSVMHEALHNHYTQKSLSLSPGK

SEQ ID NO: 44 - protein, 107 aa, Artificial Sequence; identical to SEQ ID NO: 29
  Description of Artificial Sequence: Synthetic polypeptide